European Patent Specification EP 3 472 304 B1, published August 9, 2023. Title: A NOVEL AND EFFICIENT METHOD FOR REPROGRAMMING BLOOD TO INDUCED PLURIPOTENT STEM CELLS. Applicant: CEDARS-SINAI MEDICAL CENTER SAREEN, Dhruv ORNELAS, Loren A. SVENDSEN, Clive. The sequence listing filed with the application follows.

SEQUENCE LISTING (48 sequences)

SEQ ID NO: 1 - DNA, 23 bp, Homo sapiens
ccccagggccccattttggtacc

SEQ ID NO: 2 - DNA, 26 bp, Homo sapiens
acctcagtttgaatgcatgggagagc

SEQ ID NO: 3 - DNA, 20 bp, Homo sapiens
cattcaaactgaggtaaggg

SEQ ID NO: 4 - DNA, 22 bp, Homo sapiens
tagcgtaaaaggagcaacatag

SEQ ID NO: 5 - DNA, 24 bp, Homo sapiens
ttcacatgtcccagcactaccaga

SEQ ID NO: 6 - DNA, 26 bp, Homo sapiens
tcacatgtgtgagaggggcagtgtgc

SEQ ID NO: 7 - DNA, 24 bp, Homo sapiens
ttcacatgtcccagcactaccaga

SEQ ID NO: 8 - DNA, 22 bp, Homo sapiens
tttgtttgacaggagcgacaat

SEQ ID NO: 9 - DNA, 24 bp, Homo sapiens
acccatccttcctgcccgatcaga

SEQ ID NO: 10 - DNA, 24 bp, Homo sapiens
ttggtaatggagcggcgggacttg

SEQ ID NO: 11 - DNA, 23 bp, Homo sapiens
ccacctcgccttacacatgaaga

SEQ ID NO: 12 - DNA, 22 bp, Homo sapiens
tagcgtaaaaggagcaacatag

SEQ ID NO: 13 - DNA, 26 bp, Homo sapiens
gcgaacccaagacccaggcctgctcc

SEQ ID NO: 14 - DNA, 25 bp, Homo sapiens
cagggggtctgctcgcaccgtgatg

SEQ ID NO: 15 - DNA, 21 bp, Homo sapiens
ggctgagaagaggatggctac

SEQ ID NO: 16 - DNA, 22 bp, Homo sapiens
tttgtttgacaggagcgacaat

SEQ ID NO: 17 - DNA, 25 bp, Homo sapiens
agccatatggtagcctcatgtccgc

SEQ ID NO: 18 - DNA, 30 bp, Homo sapiens
tcaattctgtgcctccgggagcagggtagg

SEQ ID NO: 19 - DNA, 25 bp, Homo sapiens
agccatatggtagcctcatgtccgc

SEQ ID NO: 20 - DNA, 22 bp, Homo sapiens
tagcgtaaaaggagcaacatag

SEQ ID NO: 21 - DNA, 21 bp, Homo sapiens
cctggaggagaagaggaaaga

SEQ ID NO: 22 - DNA, 21 bp, Homo sapiens
ttgaggacctctgtgtatttg

SEQ ID NO: 23 - DNA, 21 bp, Homo sapiens
tgctgtctccatgtttgatgt

SEQ ID NO: 24 - DNA, 21 bp, Homo sapiens
tctctgctccccacctctaag

SEQ ID NO: 25 - DNA, 21 bp, Homo sapiens
atcagggccaagacatagaga

SEQ ID NO: 26 - DNA, 20 bp, Homo sapiens
gccaatgcaacttggacgtt

SEQ ID NO: 27 - DNA, 24 bp, Homo sapiens
catagaagaagaagaggatgaaga

SEQ ID NO: 28 - DNA, 24 bp, Homo sapiens
gtagggattcgagggaattactga

SEQ ID NO: 29 - DNA, 19 bp, Homo sapiens
atggaacacgaccttgaga

SEQ ID NO: 30 - DNA, 20 bp, Homo sapiens
tgagcaggatgaggtctagg

SEQ ID NO: 31 - DNA, 20 bp, Homo sapiens
cacctcaacctggagacaat

SEQ ID NO: 32 - DNA, 20 bp, Homo sapiens
tgaagcaggcgtggtttcaa

SEQ ID NO: 33 - DNA, 20 bp, Homo sapiens
tcgggggtgttagagacaac

SEQ ID NO: 34 - DNA, 20 bp, Homo sapiens
ttccacgagggtagtgaacc

SEQ ID NO: 35 - DNA, 20 bp, Homo sapiens
accacagtccatgccatcac

SEQ ID NO: 36 - DNA, 20 bp, Homo sapiens
tccaccaccctgttgctgta

SEQ ID NO: 37 - DNA, 20 bp, Homo sapiens
tccttctacggacggaactg

SEQ ID NO: 38 - DNA, 20 bp, Homo sapiens
agaaatgcctgaggaaagca

SEQ ID NO: 39 - DNA, 20 bp, Homo sapiens
gattcctcctccaccctcac

SEQ ID NO: 40 - DNA, 23 bp, Homo sapiens
caatattctgcctggcctggatg

SEQ ID NO: 41 - DNA, 21 bp, Homo sapiens
ccacacccactcagagccatt

SEQ ID NO: 42 - DNA, 20 bp, Homo sapiens
caccccaccaccaaaacctt

SEQ ID NO: 43 - DNA, 24 bp, Homo sapiens
cgagaggaccccgtggatgcagag

SEQ ID NO: 44 - DNA, 24 bp, Homo sapiens
ggcggccatcttcagcttctccag

SEQ ID NO: 45 - DNA, 28 bp, Homo sapiens
gaatgctgcaaactgaccacgctggaac

SEQ ID NO: 46 - DNA, 28 bp, Homo sapiens
tggcattcaagagggttttcagtctgga

SEQ ID NO: 47 - DNA, 18 bp, Homo sapiens
ctatcatgctggctgcct

SEQ ID NO: 48 - DNA, 20 bp, Homo sapiens
ctacaacacccttctcacag